European Patent Application EP 4 186 522 A1, published May 31, 2023. Title: PD-L1/LAG-3 BISPECIFIC ANTIBODY FORMULATION AND PREPARATION METHOD THEREFOR AND USE THEREOF. Applicant: INNOVENT BIOLOGICS (SUZHOU) CO., LTD. The sequence listing filed with the application follows.

SEQUENCE LISTING (19 sequences)

SEQ ID NO: 1 - protein, 591 aa, Artificial Sequence
  VH-CH1-Fc-X-VHH
QLQLQESGPGLVKPSETLSLTCTVSGGSIYSESYYWGWIRQPPGKGLEWIGSIVYSGYTYYNPSLKSRVTISVDTSKNQFSLKLSSVTAADTAVYYCARVRTWDAAFDIWGQGTMVTVSSASTKGPSVFPLAPSSKSTSGGTAALGCLVKDYFPEPVTVSWNSGALTSGVHTFPAVLQSSGLYSLSSVVTVPSSSLGTQTYICNVNHKPSNTKVDKKVEPKSCDKTHTCPPCPAPEAAGGPSVFLFPPKPKDTLMISRTPEVTCVVVDVSHEDPEVKFNWYVDGVEVHNAKTKPREEQYNSTYRVVSVLTVLHQDWLNGKEYKCKVSNKALPAPIEKTISKAKGQPREPQVYTLPPSRDELTKNQVSLTCLVKGFYPSDIAVEWESNGQPENNYKTTPPVLDSDGSFFLYSKLTVDKSRWQQGNVFSCSVMHEALHNHYTQKSLSLSPGGGGGSGGGGSQVQLQESGGGLVQPGGSLRLSCAASAYTISRNSMGWFRQAPGKGLEGVAAIESDGSTSYSDSVKGRFTISLDNSKNTLYLEMNSLRAEDTAVYYCAAPKVGLGPRTALGHLAFMTLPALNYWGQGTLVTVSS

SEQ ID NO: 2 - protein, 120 aa, Artificial Sequence
  anti-LAG3 antibody VH
QLQLQESGPGLVKPSETLSLTCTVSGGSIYSESYYWGWIRQPPGKGLEWIGSIVYSGYTYYNPSLKSRVTISVDTSKNQFSLKLSSVTAADTAVYYCARVRTWDAAFDIWGQGTMVTVSS

SEQ ID NO: 3 - protein, 108 aa, Artificial Sequence
  CH1
ASTKGPSVFPLAPSSKSTSGGTAALGCLVKDYFPEPVTVSWNSGALTSGVHTFPAVLQSSGLYSLSSVVTVPSSSLGTQTYICNVNHKPSNTKVDKKVEPKSCDKTHT

SEQ ID NO: 4 - protein, 221 aa, Artificial Sequence
  Fc
CPPCPAPEAAGGPSVFLFPPKPKDTLMISRTPEVTCVVVDVSHEDPEVKFNWYVDGVEVHNAKTKPREEQYNSTYRVVSVLTVLHQDWLNGKEYKCKVSNKALPAPIEKTISKAKGQPREPQVYTLPPSRDELTKNQVSLTCLVKGFYPSDIAVEWESNGQPENNYKTTPPVLDSDGSFFLYSKLTVDKSRWQQGNVFSCSVMHEALHNHYTQKSLSLSPG

SEQ ID NO: 5 - protein, 10 aa, Artificial Sequence
  linker
GGGGSGGGGS

SEQ ID NO: 6 - protein, 132 aa, Artificial Sequence
  anti-PD-L1 single domain antibody
QVQLQESGGGLVQPGGSLRLSCAASAYTISRNSMGWFRQAPGKGLEGVAAIESDGSTSYSDSVKGRFTISLDNSKNTLYLEMNSLRAEDTAVYYCAAPKVGLGPRTALGHLAFMTLPALNYWGQGTLVTVSS

SEQ ID NO: 7 - protein, 215 aa, Artificial Sequence
  VL-CL
DIQMTQSPSSLSASVGDRVTITCQASQDISNYLNWYQQKPGKAPKLLIYDASNLETGVPSRFSGSGSGTDFTFTISSLQPEDIATYYCQQVLELPPWTFGGGTKVEIKRTVAAPSVFIFPPSDEQLKSGTASVVCLLNNFYPREAKVQWKVDNALQSGNSQESVTEQDSKDSTYSLSSTLTLSKADYEKHKVYACEVTHQGLSSPVTKSFNRGEC

SEQ ID NO: 8 - protein, 108 aa, Artificial Sequence
  anti-LAG3 antibody VL
DIQMTQSPSSLSASVGDRVTITCQASQDISNYLNWYQQKPGKAPKLLIYDASNLETGVPSRFSGSGSGTDFTFTISSLQPEDIATYYCQQVLELPPWTFGGGTKVEIK

SEQ ID NO: 9 - protein, 107 aa, Artificial Sequence [sequence omitted]

SEQ ID NO: 10 - protein, 10 aa, Artificial Sequence
  anti-PD-L1 single domain antibody CDR1
AYTISRNSMG

SEQ ID NO: 11 - protein, 16 aa, Artificial Sequence
  anti-PD-L1 single domain antibody CDR2
AIESDGSTSYSDSVKG

SEQ ID NO: 12 - protein, 24 aa, Artificial Sequence
  anti-PD-L1 single domain antibody CDR3
PKVGLGPRTALGHLAFMTLPALNY

SEQ ID NO: 13 - protein, 11 aa, Artificial Sequence
  anti-LAG3 antibody HCDR1
GSIYSESYYWG

SEQ ID NO: 14 - protein, 16 aa, Artificial Sequence
  anti-LAG3 antibody HCDR2
SIVYSGYTYYNPSLKS

SEQ ID NO: 15 - protein, 12 aa, Artificial Sequence
  anti-LAG3 antibody HCDR3
ARVRTWDAAFDI

SEQ ID NO: 16 - protein, 11 aa, Artificial Sequence
  anti-LAG3 antibody LCDR1
QASQDISNYLN

SEQ ID NO: 17 - protein, 7 aa, Artificial Sequence
  anti-LAG3 antibody LCDR2
DASNLET

SEQ ID NO: 18 - protein, 10 aa, Artificial Sequence
  anti-LAG3 antibody LCDR3
QQVLELPPWT

SEQ ID NO: 19 - protein, 449 aa, Artificial Sequence
  anti-LAG3 antibody heavy chain
QLQLQESGPGLVKPSETLSLTCTVSGGSIYSESYYWGWIRQPPGKGLEWIGSIVYSGYTYYNPSLKSRVTISVDTSKNQFSLKLSSVTAADTAVYYCARVRTWDAAFDIWGQGTMVTVSSASTKGPSVFPLAPSSKSTSGGTAALGCLVKDYFPEPVTVSWNSGALTSGVHTFPAVLQSSGLYSLSSVVTVPSSSLGTQTYICNVNHKPSNTKVDKKVEPKSCDKTHTCPPCPAPEAAGGPSVFLFPPKPKDTLMISRTPEVTCVVVDVSHEDPEVKFNWYVDGVEVHNAKTKPREEQYNSTYRVVSVLTVLHQDWLNGKEYKCKVSNKALPAPIEKTISKAKGQPREPQVYTLPPSRDELTKNQVSLTCLVKGFYPSDIAVEWESNGQPENNYKTTPPVLDSDGSFFLYSKLTVDKSRWQQGNVFSCSVMHEALHNHYTQKSLSLSPG